European Patent Application EP 4 471 145 A1, published December 4, 2024. Title: 小RNA及其在高血脂治疗中的用途. Applicant: 中国医学科学院基础医学研究所. Application CN. The sequence listing filed with the application follows.

SEQUENCE LISTING (77 sequences)

SEQ ID NO: 1 - RNA, 18 nt, Artificial Sequence
  source 1..18: mol_type = unassigned RNA
agcagcagcagcagcagc

SEQ ID NO: 2 - RNA, 19 nt, Artificial Sequence
  source 1..19: mol_type = unassigned RNA
agcagcagcagcagcagca

SEQ ID NO: 3 - RNA, 20 nt, Artificial Sequence
  source 1..20: mol_type = unassigned RNA
agcagcagcagcagcagcag

SEQ ID NO: 4 - RNA, 18 nt, Artificial Sequence
  source 1..18: mol_type = unassigned RNA
cagcagcagcagcagcag

SEQ ID NO: 5 - RNA, 19 nt, Artificial Sequence
  source 1..19: mol_type = unassigned RNA
cagcagcagcagcagcagc

SEQ ID NO: 6 - RNA, 20 nt, Artificial Sequence
  source 1..20: mol_type = unassigned RNA
cagcagcagcagcagcagca

SEQ ID NO: 7 - RNA, 21 nt, Artificial Sequence
  misc_feature 1..21
  source 1..21: mol_type = unassigned RNA
cagcagcagcagcagcagcag

SEQ ID NO: 8 - RNA, 21 nt, (Artificial Sequence)
  misc_feature 1..21: note = PCSK9-sRNA-27
  source 1..21: mol_type = unassigned RNA
tcgacgcgggctctgctcgtt

SEQ ID NO: 9 - RNA, 21 nt, (Artificial Sequence)
  misc_feature 1..21: note = PCSK9-sRNA-28
  source 1..21: mol_type = unassigned RNA
ccgtgcgctggattatgactg

SEQ ID NO: 10 - RNA, 21 nt, (Artificial Sequence)
  misc_feature 1..21: note = PCSK9-sRNA-29
  source 1..21: mol_type = unassigned RNA
tgggcggcattgtctgcggat

SEQ ID NO: 11 - RNA, 21 nt, (Artificial Sequence)
  misc_feature 1..21: note = PCSK9-sRNA-30
  source 1..21: mol_type = unassigned RNA
tgcagccccaatcgggcggta

SEQ ID NO: 12 - RNA, 21 nt, (Artificial Sequence)
  misc_feature 1..21: note = PCSK9-sRNA-31
  source 1..21: mol_type = unassigned RNA
tgcggctggatcacctccttt

SEQ ID NO: 13 - RNA, 21 nt, (Artificial Sequence)
  misc_feature 1..21: note = PCSK9-sRNA-32
  source 1..21: mol_type = unassigned RNA
cgcgcttgactgcgagacaga

SEQ ID NO: 14 - RNA, 21 nt, (Artificial Sequence)
  misc_feature 1..21: note = PCSK9-sRNA-33
  source 1..21: mol_type = unassigned RNA
atggctgtcgtcagctcgtgt

SEQ ID NO: 15 - RNA, 21 nt, (Artificial Sequence)
  misc_feature 1..21: note = PCSK9-sRNA-36
  source 1..21: mol_type = unassigned RNA
ccggcggactgctcgagctgc

SEQ ID NO: 16 - RNA, 21 nt, (Artificial Sequence)
  misc_feature 1..21: note = PCSK9-sRNA-39
  source 1..21: mol_type = unassigned RNA
ctgccggcggactgctcgagc

SEQ ID NO: 17 - RNA, 21 nt, (Artificial Sequence)
  misc_feature 1..21: note = PCSK9-sRNA-40
  source 1..21: mol_type = unassigned RNA
cccagccccgaacccgtcggc

SEQ ID NO: 18 - RNA, 21 nt, (Artificial Sequence)
  misc_feature 1..21: note = PCSK9-sRNA-41
  source 1..21: mol_type = unassigned RNA
cggctgtcggtggtctgctcg

SEQ ID NO: 19 - RNA, 21 nt, (Artificial Sequence)
  misc_feature 1..21: note = PCSK9-sRNA-55
  source 1..21: mol_type = unassigned RNA
ggtggctgtagtttagtggta

SEQ ID NO: 20 - RNA, 21 nt, (Artificial Sequence)
  misc_feature 1..21: note = PCSK9-sRNA-58
  source 1..21: mol_type = unassigned RNA
agcttcagttgtccgatttgt

SEQ ID NO: 21 - RNA, 21 nt, (Artificial Sequence)
  misc_feature 1..21: note = PCSK9-sRNA-62
  source 1..21: mol_type = unassigned RNA
agggctgtagctcagttggta

SEQ ID NO: 22 - RNA, 21 nt, (Artificial Sequence)
  misc_feature 1..21: note = PCSK9-sRNA-63
  source 1..21: mol_type = unassigned RNA
cctcggccggatgcggaacgg

SEQ ID NO: 23 - RNA, 21 nt, (Artificial Sequence)
  misc_feature 1..21: note = PCSK9-sRNA-68
  source 1..21: mol_type = unassigned RNA
ccgaccccgatcttctgtgaa

SEQ ID NO: 24 - RNA, 21 nt, (Artificial Sequence)
  misc_feature 1..21: note = PCSK9-sRNA-71
  source 1..21: mol_type = unassigned RNA
gctcgtagttggaccttgggt

SEQ ID NO: 25 - RNA, 21 nt, (Artificial Sequence)
  misc_feature 1..21: note = PCSK9-sRNA-72
  source 1..21: mol_type = unassigned RNA
gctcgtagttggaccttggga

SEQ ID NO: 26 - RNA, 21 nt, (Artificial Sequence)
  misc_feature 1..21: note = PCSK9-sRNA-75
  source 1..21: mol_type = unassigned RNA
ccctgcgtcgctccgattcgt

SEQ ID NO: 27 - RNA, 21 nt, (Artificial Sequence)
  misc_feature 1..21: note = PCSK9-sRNA-77
  source 1..21: mol_type = unassigned RNA
tcttcggaatttgaagctaga

SEQ ID NO: 28 - RNA, 21 nt, (Artificial Sequence)
  misc_feature 1..21: note = PCSK9-sRNA-79
  source 1..21: mol_type = unassigned RNA
tcctcgatggtctaacggtca

SEQ ID NO: 29 - RNA, 21 nt, (Artificial Sequence)
  misc_feature 1..21: note = PCSK9-sRNA-80
  source 1..21: mol_type = unassigned RNA
cggctgtcggcgaactgctcg

SEQ ID NO: 30 - RNA, 21 nt, (Artificial Sequence)
  misc_feature 1..21: note = PCSK9-sRNA-81
  source 1..21: mol_type = unassigned RNA
acacggtccagactcctacgg

SEQ ID NO: 31 - RNA, 21 nt, (Artificial Sequence)
  misc_feature 1..21: note = PCSK9-sRNA-82
  source 1..21: mol_type = unassigned RNA
cgtttcacgtcgggttcacca

SEQ ID NO: 32 - RNA, 21 nt, (Artificial Sequence)
  misc_feature 1..21: note = PCSK9-sRNA-83
  source 1..21: mol_type = unassigned RNA
aatggcaccgtaacttcggga

SEQ ID NO: 33 - RNA, 21 nt, (Artificial Sequence)
  misc_feature 1..21: note = PCSK9-sRNA-84
  source 1..21: mol_type = unassigned RNA
cggaagccgggttacggtgcc

SEQ ID NO: 34 - RNA, 21 nt, (Artificial Sequence)
  misc_feature 1..21: note = PCSK9-sRNA-85
  source 1..21: mol_type = unassigned RNA
cgccgtccgaattgtagtctg

SEQ ID NO: 35 - RNA, 21 nt, (Artificial Sequence)
  misc_feature 1..21: note = PCSK9-sRNA-86
  source 1..21: mol_type = unassigned RNA
tggctgtcgtcagctcgtgtt

SEQ ID NO: 36 - RNA, 21 nt, (Artificial Sequence)
  misc_feature 1..21: note = PCSK9-sRNA-87
  source 1..21: mol_type = unassigned RNA
cggaatccgctaaggactgtg

SEQ ID NO: 37 - RNA, 21 nt, (Artificial Sequence)
  misc_feature 1..21: note = PCSK9-sRNA-88
  source 1..21: mol_type = unassigned RNA
tgcgcctcggtcggatgtgga

SEQ ID NO: 38 - RNA, 21 nt, (Artificial Sequence)
  misc_feature 1..21: note = PCSK9-sRNA-90
  source 1..21: mol_type = unassigned RNA
ctccccatccggcccgtcttg

SEQ ID NO: 39 - RNA, 21 nt, (Artificial Sequence)
  misc_feature 1..21: note = PCSK9-sRNA-91
  source 1..21: mol_type = unassigned RNA
ccggtgcgttcctgacagtct

SEQ ID NO: 40 - RNA, 21 nt, (Artificial Sequence)
  misc_feature 1..21: note = PCSK9-sRNA-93
  source 1..21: mol_type = unassigned RNA
tgcctggcggctgtagcgcgg

SEQ ID NO: 41 - RNA, 21 nt, (Artificial Sequence)
  misc_feature 1..21: note = PCSK9-sRNA-94
  source 1..21: mol_type = unassigned RNA
cgaatcctggctgttgtatgt

SEQ ID NO: 42 - RNA, 21 nt, (Artificial Sequence)
  misc_feature 1..21: note = PCSK9-sRNA-95
  source 1..21: mol_type = unassigned RNA
catgcctgtccgagcgtcatt

SEQ ID NO: 43 - RNA, 21 nt, (Artificial Sequence)
  misc_feature 1..21: note = PCSK9-sRNA-96
  source 1..21: mol_type = unassigned RNA
catgcctgttcgagcgtcatt

SEQ ID NO: 44 - RNA, 21 nt, (Artificial Sequence)
  misc_feature 1..21: note = PCSK9-sRNA-98
  source 1..21: mol_type = unassigned RNA
atcggctcgggacattgaccg

SEQ ID NO: 45 - RNA, 21 nt, (Artificial Sequence)
  misc_feature 1..21: note = PCSK9-sRNA-99
  source 1..21: mol_type = unassigned RNA
tattctggtgtcctaggcgta

SEQ ID NO: 46 - RNA, 21 nt, (Artificial Sequence)
  misc_feature 1..21: note = PCSK9-sRNA-100
  source 1..21: mol_type = unassigned RNA
ccttcggagtttgaagctaga

SEQ ID NO: 47 - RNA, 21 nt, (Artificial Sequence)
  misc_feature 1..21: note = PCSK9-sRNA-101
  source 1..21: mol_type = unassigned RNA
cggactgctcgagctgcttcc

SEQ ID NO: 48 - RNA, 21 nt, (Artificial Sequence)
  misc_feature 1..21: note = PCSK9-sRNA-102
  source 1..21: mol_type = unassigned RNA
atgcgagagtagggaactgcc

SEQ ID NO: 49 - RNA, 21 nt, (Artificial Sequence)
  misc_feature 1..21: note = PCSK9-sRNA-103
  source 1..21: mol_type = unassigned RNA
cttgactctagtccgactttg

SEQ ID NO: 50 - RNA, 21 nt, (Artificial Sequence)
  misc_feature 1..21: note = PCSK9-sRNA-104
  source 1..21: mol_type = unassigned RNA
atcgactcggggcgtggaccg

SEQ ID NO: 51 - RNA, 21 nt, (Artificial Sequence)
  misc_feature 1..21: note = PCSK9-sRNA-107
  source 1..21: mol_type = unassigned RNA
gtggctgtagtttagtggtaa

SEQ ID NO: 52 - RNA, 21 nt, (Artificial Sequence)
  misc_feature 1..21: note = PCSK9-sRNA-109
  source 1..21: mol_type = unassigned RNA
gctcgtagttggactttgggt

SEQ ID NO: 53 - RNA, 21 nt, (Artificial Sequence)
  misc_feature 1..21: note = PCSK9-sRNA-110
  source 1..21: mol_type = unassigned RNA
gctcgtagttggactttggga

SEQ ID NO: 54 - RNA, 21 nt, (Artificial Sequence)
  misc_feature 1..21: note = PCSK9-sRNA-111
  source 1..21: mol_type = unassigned RNA
tcctcgatggtctaacggcta

SEQ ID NO: 55 - RNA, 21 nt, (Artificial Sequence)
  misc_feature 1..21: note = PCSK9-sRNA-112
  source 1..21: mol_type = unassigned RNA
cgggctttgcccggtgctctg

SEQ ID NO: 56 - RNA, 21 nt, (Artificial Sequence)
  misc_feature 1..21: note = PCSK9-sRNA-113
  source 1..21: mol_type = unassigned RNA
tgtgagctcgatgagtagggc

SEQ ID NO: 57 - RNA, 21 nt, (Artificial Sequence)
  misc_feature 1..21: note = PCSK9-sRNA-114
  source 1..21: mol_type = unassigned RNA
acacggcccagactcctacgg

SEQ ID NO: 58 - RNA, 21 nt, (Artificial Sequence)
  misc_feature 1..21: note = PCSK9-sRNA-115
  source 1..21: mol_type = unassigned RNA
gtggagcggtgaaatgcgtag

SEQ ID NO: 59 - RNA, 21 nt, (Artificial Sequence)
  misc_feature 1..21: note = PCSK9-sRNA-116
  source 1..21: mol_type = unassigned RNA
cccgtcggctgtcggtggact

SEQ ID NO: 60 - RNA, 21 nt, (Artificial Sequence)
  misc_feature 1..21: note = PCSK9-sRNA-117
  source 1..21: mol_type = unassigned RNA
taggtagcgcctcatgtatca

SEQ ID NO: 61 - RNA, 21 nt, (Artificial Sequence)
  misc_feature 1..21: note = PCSK9-sRNA-118
  source 1..21: mol_type = unassigned RNA
cgattctcggattggacacca

SEQ ID NO: 62 - RNA, 21 nt, (Artificial Sequence)
  misc_feature 1..21: note = PCSK9-sRNA-119
  source 1..21: mol_type = unassigned RNA
ctcactggtcgagtcggcctg

SEQ ID NO: 63 - RNA, 21 nt, (Artificial Sequence)
  misc_feature 1..21: note = PCSK9-sRNA-122
  source 1..21: mol_type = unassigned RNA
attccggtcctattctgttgg

SEQ ID NO: 64 - RNA, 21 nt, (Artificial Sequence)
  misc_feature 1..21: note = PCSK9-sRNA-123
  source 1..21: mol_type = unassigned RNA
gtgttgacttcagttttatga

SEQ ID NO: 65 - RNA, 21 nt, (Artificial Sequence)
  misc_feature 1..21: note = PCSK9-sRNA-124
  source 1..21: mol_type = unassigned RNA
aggacgtgctaatctgcgaaa

SEQ ID NO: 66 - RNA, 21 nt, (Artificial Sequence)
  misc_feature 1..21: note = PCSK9-sRNA-125
  source 1..21: mol_type = unassigned RNA
aaagttgggggctcgaagacg

SEQ ID NO: 67 - RNA, 21 nt, (Artificial Sequence)
  misc_feature 1..21: note = PCSK9-sRNA-126
  source 1..21: mol_type = unassigned RNA
atgcctgtttgagcgtcattt

SEQ ID NO: 68 - RNA, 21 nt, (Artificial Sequence)
  misc_feature 1..21: note = PCSK9-sRNA-127
  source 1..21: mol_type = unassigned RNA
cggctggatcacctcctttct

SEQ ID NO: 69 - RNA, 21 nt, (Artificial Sequence)
  misc_feature 1..21: note = PCSK9-sRNA-131
  source 1..21: mol_type = unassigned RNA
cggacaaggggaatccgactg

SEQ ID NO: 70 - RNA, 21 nt, (Artificial Sequence)
  misc_feature 1..21: note = PCSK9-sRNA-132
  source 1..21: mol_type = unassigned RNA
cgcctcgtgaactcatcttcg

SEQ ID NO: 71 - RNA, 21 nt, (Artificial Sequence)
  misc_feature 1..21: note = PCSK9-sRNA-135
  source 1..21: mol_type = unassigned RNA
ccccatgccgcaccgattcgt

SEQ ID NO: 72 - RNA, 21 nt, (Artificial Sequence)
  misc_feature 1..21: note = PCSK9-sRNA-136
  source 1..21: mol_type = unassigned RNA
tcctgtactgagctgccccga

SEQ ID NO: 73 - RNA, 21 nt, (Artificial Sequence)
  misc_feature 1..21: note = PCSK9-sRNA-137
  source 1..21: mol_type = unassigned RNA
gcaccggctaactctgtgcca

SEQ ID NO: 74 - RNA, 26 nt, Artificial Sequence
  source 1..26: mol_type = unassigned RNA
gcctgggcggagcggtcgtcggtgca

SEQ ID NO: 75 - RNA, 21 nt, Artificial Sequence
  source 1..21: mol_type = unassigned RNA
tgcagccccaatagggcggta

SEQ ID NO: 76 - DNA, 21 bp, Homo sp.
  source 1..21: mol_type = genomic DNA
ctgctgctgctgctgctgctg

SEQ ID NO: 77 - DNA, 21 bp, Homo sp.
  source 1..21: mol_type = genomic DNA
ctgctgttgctgctgctgctg